European Patent Application EP 4 186 972 A1, published May 31, 2023. Title: CONTROLLABLE TRANSCRIPTION. Applicant: Cambridge Enterprise Limited. Application EP. The sequence listing filed with the application follows.

SEQUENCE LISTING (86 sequences)

SEQ ID NO: 1 - DNA, 19 bp, synthetic construct
  misc_feature 1..19: note = TetO2 19 nucleotide sequence
  source 1..19: mol_type = other DNA
tccctatcagtgatagaga

SEQ ID NO: 2 - DNA, 1797 bp, Homo sapiens
  source 1..1797: mol_type = genomic DNA
gctcgaaaccggacggagccattgctctcgcagagggaggagcgcttccggctagcctcttgtcgccgattggccgtttctcctcccgccgtgtgtgaaaacacaaatggcgtattctggttggagtaaagctcctgtcagttacgccgtcgggagtacgcagccgcttagcgactctcgcgttgccccctgggtggggcgggtaggtaggtggggtgtagagatgctgggtgtgcgggcgcggccggcctcctgcggcgggaggggagggtcagtgaaatcggctctggcgcgggcgtcctcccaccctccccttccttcgggggagtcggtttacccgccgcctgcttgtcttcgacacctgattggctgtcgaagctgtgggaccgggcccttgctactggctcgagtctcacatgagcgaaaccactgcgcggggcgcgggggtggcggggaggcgggcgttggtacggtcctccccgaggccgagcgccgcagtgtctggccccgcgcccctgcgcaacgtggcaggaagcgcgcgctggaggcgggggcgggctgccggccgagacttctggatggcggcggccgcggctccgccccgggttcccaccgcctgaagggcgagacaagcccgacctgctacaggcactcgtgggggtgggggaggagcgggggtcggtccggctggtttgtgggtgggaggcgcttgttctccaaaaaccggcgcgagctgcaatcctgagggagctgcggtggaggaggtggagagaaggccgcacccttctgggcagggggaggggagtgccgcaatacctttatgggagttctctgctgcctcccgtcttgtaaggaccgccctgggcctggaagaagccctccctcctttcctcctcgcgtgatctcgtcatcgcctccatgtcgagtcgcttctcgattatgggcgggattcttttgcctaggcttaaggggctaacttggtccctgggcgttgccctgcaggggagtgagcagctgtaagatttgaggggcgactccgattagtttatcttcccacggactagagttggtgtcgaggttattgtaataagggtggggtagggaaatggagcttagtcattcacctggggctgattttatgcaacgagactgcggattatcactacttatcatttttggagcatttttctagagacagacataaagcatgatcacctgagttttataccatttgagacccttgctgcaccaccaaagtgtagcatcaggttaaatcttaatagaaaaattttagcttttgcttgagaaaccagtgcttccctccctcaccctctctccccaggctctctacccctttgcatccctaccaggcatcttagcaactctcactcatacttgatcccattttccatttgttgtacttgctcctctagtattcagacatagcactagctttctccctctcttgatcttgggtagcctggtgtctcgcgaaaccagacagattggttccaccacaaattaaggcttgagctggggcttgactcttacccagcagtgcttttattcctccctagttcacgttcttaaatgtttatcttgattttcattttatcctttttccttagctgggattctgtccctgaccgtcttcacagtccaggtgatcttgactactgctttacagagaattggatctgaggttaggcaacatctccctttttcttcctctaaatacctctcatttctgttcttaccagttagtaactgatctcagatgcctgtgtgatagcttcc

SEQ ID NO: 3 - DNA, 651 bp, synthetic construct
  misc_feature 1..651: note = STDtetR-nls
  source 1..651: mol_type = other DNA
atgccaaaaaagaagaggaaggtatctagattagataaaagtaaagtgattaacagcgcattagagctgcttaatgaggtcggaatcgaaggtttaacaacccgtaaactcgcccagaagctaggtgtagagcagcctacattgtattggcatgtaaaaaataagcgggctttgctcgacgccttagccattgagatgttagataggcaccatactcacttttgccctttagaaggggaaagctggcaagattttttacgtaataacgctaaaagttttagatgtgctttactaagtcatcgcgatggagcaaaagtacatttaggtacacggcctacagaaaaacagtatgaaactctcgaaaatcaattagcctttttatgccaacaaggtttttcactagagaatgcattatatgcactcagcgctgtggggcattttactttaggttgcgtattggaagatcaagagcatcaagtcgctaaagaagaaagggaaacacctactactgatagtatgccgccattattacgacaagctatcgaattatttgatcaccaaggtgcagagccagccttcttattcggccttgaattgatcatatgcggattagaaaaacaacttaaatgtgaaagtgggtctccgcggtaa

SEQ ID NO: 4 - protein, 216 aa, synthetic construct [sequence omitted]

SEQ ID NO: 5 - DNA, 651 bp, synthetic construct
  misc_feature 1..651: note = OPTtetR
  source 1..651: mol_type = other DNA
atgcccaagaaaaagcggaaggtgtcccggctggacaagagcaaagtgatcaacagcgccctggaactgctgaacgaagtgggcatcgagggcctgaccacccggaagctggcccagaaactgggcgtggaacagcccaccctgtactggcacgtgaagaacaagcgggccctgctggacgccctggccatcgagatgctggaccggcaccacacacacttttgccccctggaaggcgaaagctggcaggacttcctgcggaacaacgccaagagcttcagatgcgccctgctgagccaccgggacggcgccaaagtgcacctgggcaccagacccaccgagaagcagtacgagacactggaaaaccagctggccttcctgtgccagcagggcttcagcctggaaaacgccctgtacgccctgagcgccgtgggccactttaccctgggctgcgtgctggaagatcaggaacaccaggtcgccaaagaggaaagagagacacccaccaccgacagcatgccccccctgctgagacaggccatcgagctgttcgatcatcaaggcgccgagcccgccttcctgttcggcctggaactgatcatctgcggcctcgagaagcagctgaagtgcgagagcggctcccccagatga

SEQ ID NO: 6 - protein, 216 aa, synthetic construct [sequence omitted]

SEQ ID NO: 7 - DNA, 20 bp, synthetic construct
  misc_feature 1..20: note = hROSA26 Locus PCR
  source 1..20: mol_type = other DNA
gagaagaggctgtgcttcgg

SEQ ID NO: 8 - DNA, 22 bp, synthetic construct
  misc_feature 1..22: note = hROSA26 Locus PCR
  source 1..22: mol_type = other DNA
acagtacaagccagtaatggag

SEQ ID NO: 9 - DNA, 20 bp, synthetic construct
  misc_feature 1..20: note = hROSA26 5'-INT PCR
  source 1..20: mol_type = other DNA
gagaagaggctgtgcttcgg

SEQ ID NO: 10 - DNA, 21 bp, synthetic construct
  misc_feature 1..21: note = hROSA26 5'-INT PCR
  source 1..21: mol_type = other DNA
aagaccgcgaagagtttgtcc

SEQ ID NO: 11 - DNA, 21 bp, synthetic construct
  misc_feature 1..21: note = hROSA26 3'-INT PCR
  source 1..21: mol_type = other DNA
gaaactcgctcaaaagctggg

SEQ ID NO: 12 - DNA, 22 bp, synthetic construct
  misc_feature 1..22: note = hROSA26 3'-INT PCR
  source 1..22: mol_type = other DNA
acagtacaagccagtaatggag

SEQ ID NO: 13 - DNA, 21 bp, synthetic construct
  misc_feature 1..21: note = hROSA26 3'-BB PCR
  source 1..21: mol_type = other DNA
gaaactcgctcaaaagctggg

SEQ ID NO: 14 - DNA, 20 bp, synthetic construct
  misc_feature 1..20: note = hROSA26 3'-BB PCR
  source 1..20: mol_type = other DNA
tgaccatgattacgccaagc

SEQ ID NO: 15 - DNA, 25 bp, synthetic construct
  misc_feature 1..25: note = AAVS1 Locus PCR
  source 1..25: mol_type = other DNA
ctgtttccccttcccaggcaggtcc

SEQ ID NO: 16 - DNA, 25 bp, synthetic construct
  misc_feature 1..25: note = AAVS1 Locus PCR
  source 1..25: mol_type = other DNA
tgcaggggaacggggctcagtctga

SEQ ID NO: 17 - DNA, 25 bp, synthetic construct
  misc_feature 1..25: note = AAVS1 5'-INT PCR
  source 1..25: mol_type = other DNA
ctgtttccccttcccaggcaggtcc

SEQ ID NO: 18 - DNA, 25 bp, synthetic construct
  misc_feature 1..25: note = AAVS1 5'-INT PCR
  source 1..25: mol_type = other DNA
tcgtcgcgggtggcgaggcgcaccg

SEQ ID NO: 19 - DNA, 25 bp, synthetic construct
  misc_feature 1..25: note = AAVS1 3'-INT PCR
  source 1..25: mol_type = other DNA
tgcaggggaacggggctcagtctga

SEQ ID NO: 20 - DNA, 20 bp, synthetic construct
  misc_feature 1..20: note = AAVS1 3'-BB PCR
  source 1..20: mol_type = other DNA
atgcttccggctcgtatgtt

SEQ ID NO: 21 - DNA, 22 bp, synthetic construct
  misc_feature 1..22: note = CNP Fw
  source 1..22: mol_type = other DNA
tcctcatcatgaacagaggctt

SEQ ID NO: 22 - DNA, 20 bp, synthetic construct
  misc_feature 1..20: note = CNP Rev
  source 1..20: mol_type = other DNA
aaactgcagctcaggcttgt

SEQ ID NO: 23 - DNA, 20 bp, synthetic construct
  misc_feature 1..20: note = DES Fw
  source 1..20: mol_type = other DNA
ccaacaagaacaacgacgcc

SEQ ID NO: 24 - DNA, 21 bp, synthetic construct
  misc_feature 1..21: note = DES Rev
  source 1..21: mol_type = other DNA
atcagggaatcgttagtgccc

SEQ ID NO: 25 - DNA, 22 bp, synthetic construct
  misc_feature 1..22: note = DMD Fw
  source 1..22: mol_type = other DNA
tggtgggaagaagtagaggact

SEQ ID NO: 26 - DNA, 20 bp, synthetic construct
  misc_feature 1..20: note = DMD Rev
  source 1..20: mol_type = other DNA
tgctgcttcccaaacttaga

SEQ ID NO: 27 - DNA, 20 bp, synthetic construct
  misc_feature 1..20: note = EGFP Fw
  source 1..20: mol_type = other DNA
cccgacaaccactacctgag

SEQ ID NO: 28 - DNA, 20 bp, synthetic construct
  misc_feature 1..20: note = EGFP Rev
  source 1..20: mol_type = other DNA
gtccatgccgagagtgatcc

SEQ ID NO: 29 - DNA, 20 bp, synthetic construct
  misc_feature 1..20: note = FOXG1 Fw
  source 1..20: mol_type = other DNA
tgccaagttttacgacggga

SEQ ID NO: 30 - DNA, 20 bp, synthetic construct
  misc_feature 1..20: note = FOXG1 Rev
  source 1..20: mol_type = other DNA
gggttggaagaagacccctg

SEQ ID NO: 31 - DNA, 20 bp, synthetic construct
  misc_feature 1..20: note = GRIA4 Fw
  source 1..20: mol_type = other DNA
ggccagggaattgacatgga

SEQ ID NO: 32 - DNA, 23 bp, synthetic construct
  misc_feature 1..23: note = GRIA4 Rev
  source 1..23: mol_type = other DNA
aaccaacctttctaggtcctgtg

SEQ ID NO: 33 - DNA, 20 bp, synthetic construct
  misc_feature 1..20: note = HMBS (PBGD) Fw
  source 1..20: mol_type = other DNA
attaccccgggagactgaac

SEQ ID NO: 34 - DNA, 20 bp, synthetic construct
  misc_feature 1..20: note = HMBS (PBGD) Rev
  source 1..20: mol_type = other DNA
ggctgttgcttggacttctc

SEQ ID NO: 35 - DNA, 20 bp, synthetic construct
  misc_feature 1..20: note = MAG Fw
  source 1..20: mol_type = other DNA
cagaagacgtccccaactca

SEQ ID NO: 36 - DNA, 22 bp, synthetic construct
  misc_feature 1..22: note = MAG Rev
  source 1..22: mol_type = other DNA
cctcgggaggctgaaatcataa

SEQ ID NO: 37 - DNA, 21 bp, synthetic construct
  misc_feature 1..21: note = MAP2 Fw
  source 1..21: mol_type = other DNA
agactgcagctctgcctttag

SEQ ID NO: 38 - DNA, 23 bp, synthetic construct
  misc_feature 1..23: note = MAP2 Rev
  source 1..23: mol_type = other DNA
aggctgtaagtaaatcttcctcc

SEQ ID NO: 39 - DNA, 24 bp, synthetic construct
  misc_feature 1..24: note = MBP Fw
  source 1..24: mol_type = other DNA
tggtgatggagatgtcaagcaggt

SEQ ID NO: 40 - DNA, 24 bp, synthetic construct
  misc_feature 1..24: note = MBP Rev
  source 1..24: mol_type = other DNA
gctgtggtttggaaacgaggttgt

SEQ ID NO: 41 - DNA, 23 bp, synthetic construct
  misc_feature 1..23: note = MOG Fw
  source 1..23: mol_type = other DNA
agagatagagaatctccaccgga

SEQ ID NO: 42 - DNA, 21 bp, synthetic construct
  misc_feature 1..21: note = MOG Rev
  source 1..21: mol_type = other DNA
tgatcaaggcaaccaagggtc

SEQ ID NO: 43 - DNA, 22 bp, synthetic construct
  misc_feature 1..22: note = MYH1 Fw
  source 1..22: mol_type = other DNA
cacactagtttcacagctctcg

SEQ ID NO: 44 - DNA, 20 bp, synthetic construct
  misc_feature 1..20: note = MYH1 Rev
  source 1..20: mol_type = other DNA
cagggcactcttggccttta

SEQ ID NO: 45 - DNA, 21 bp, synthetic construct
  misc_feature 1..21: note = MYH2 Fw
  source 1..21: mol_type = other DNA
ggaagctctggtgtctcagtt

SEQ ID NO: 46 - DNA, 21 bp, synthetic construct
  misc_feature 1..21: note = MYH2 Rev
  source 1..21: mol_type = other DNA
cagggcgttcttggcttttat

SEQ ID NO: 47 - DNA, 20 bp, synthetic construct
  misc_feature 1..20: note = MYH3 Fw
  source 1..20: mol_type = other DNA
gctgcatacccagaacacca

SEQ ID NO: 48 - DNA, 20 bp, synthetic construct
  misc_feature 1..20: note = MYH3 Rev
  source 1..20: mol_type = other DNA
ccctgctggcatcttctacc

SEQ ID NO: 49 - DNA, 20 bp, synthetic construct
  misc_feature 1..20: note = MYH4 Fw
  source 1..20: mol_type = other DNA
tcgcatttgtcagccaaggg

SEQ ID NO: 50 - DNA, 21 bp, synthetic construct
  misc_feature 1..21: note = MYH4 Rev
  source 1..21: mol_type = other DNA
tgaaacccaggatgtccacag

SEQ ID NO: 51 - DNA, 20 bp, synthetic construct
  misc_feature 1..20: note = MYH7 Fw
  source 1..20: mol_type = other DNA
gagactgtcgtgggcttgta

SEQ ID NO: 52 - DNA, 21 bp, synthetic construct
  misc_feature 1..21: note = MYH7 Rev
  source 1..21: mol_type = other DNA
gcccttctcaataggcgcatc

SEQ ID NO: 53 - DNA, 20 bp, synthetic construct
  misc_feature 1..20: note = MYH8 Fw
  source 1..20: mol_type = other DNA
tgaagcagatagcagcgcga

SEQ ID NO: 54 - DNA, 20 bp, synthetic construct
  misc_feature 1..20: note = MYH8 Rev
  source 1..20: mol_type = other DNA
cgtacgaagtgagggtgtgt

SEQ ID NO: 55 - DNA, 20 bp, synthetic construct
  misc_feature 1..20: note = MYOD1 (endo) Fw
  source 1..20: mol_type = other DNA
gccgctttccttaaccacaa

SEQ ID NO: 56 - DNA, 20 bp, synthetic construct
  misc_feature 1..20: note = MYOD1 (endo) Rev
  source 1..20: mol_type = other DNA
ctgaatgcccacccactgtc

SEQ ID NO: 57 - DNA, 20 bp, synthetic construct
  misc_feature 1..20: note = MYOD1 Fw
  source 1..20: mol_type = other DNA
cgacggcatgatggactaca

SEQ ID NO: 58 - DNA, 20 bp, synthetic construct
  misc_feature 1..20: note = MYOD1 Rev
  source 1..20: mol_type = other DNA
tagtaggcgccttcgtagca

SEQ ID NO: 59 - DNA, 22 bp, synthetic construct
  misc_feature 1..22: note = NANOG Fw
  source 1..22: mol_type = other DNA
agcagatgcaagaactctccaa

SEQ ID NO: 60 - DNA, 20 bp, synthetic construct
  misc_feature 1..20: note = NANOG Rev
  source 1..20: mol_type = other DNA
tgaggccttctgcgtcacac

SEQ ID NO: 61 - DNA, 21 bp, synthetic construct
  misc_feature 1..21: note = NEUROG2 (NGN2) Fw
  source 1..21: mol_type = other DNA
tgttcgtcaaatccgagacct

SEQ ID NO: 62 - DNA, 20 bp, synthetic construct
  misc_feature 1..20: note = NEUROG2 (NGN2) Rev
  source 1..20: mol_type = other DNA
cgatccgagcagcactaaca

SEQ ID NO: 63 - DNA, 20 bp, synthetic construct
  misc_feature 1..20: note = PAX6 Fw
  source 1..20: mol_type = other DNA
cgagatttcagagccccata

SEQ ID NO: 64 - DNA, 20 bp, synthetic construct
  misc_feature 1..20: note = PAX6 Rev
  source 1..20: mol_type = other DNA
aagacaccaccgagctgatt

SEQ ID NO: 65 - DNA, 22 bp, synthetic construct
  misc_feature 1..22: note = PLP Fw
  source 1..22: mol_type = other DNA
aacagctgagttccaaatgacc

SEQ ID NO: 66 - DNA, 20 bp, synthetic construct
  misc_feature 1..20: note = PLP Rev
  source 1..20: mol_type = other DNA
acggcaaagttgtaagtggc

SEQ ID NO: 67 - DNA, 20 bp, synthetic construct
  misc_feature 1..20: note = POU3F2 (BRN2) Fw
  source 1..20: mol_type = other DNA
acccgctttatcgaaggcaa

SEQ ID NO: 68 - DNA, 20 bp, synthetic construct
  misc_feature 1..20: note = POU3F2 (BRN2) Rev
  source 1..20: mol_type = other DNA
cctccataacctcccccaga

SEQ ID NO: 69 - DNA, 20 bp, synthetic construct
  misc_feature 1..20: note = POU5F1 (OCT4) Fw
  source 1..20: mol_type = other DNA
gtggaggaagctgacaacaa

SEQ ID NO: 70 - DNA, 20 bp, synthetic construct
  misc_feature 1..20: note = POU5F1 (OCT4) Rev
  source 1..20: mol_type = other DNA
attctccaggttgcctctca

SEQ ID NO: 71 - DNA, 20 bp, synthetic construct
  misc_feature 1..20: note = RYR1 Fw
  source 1..20: mol_type = other DNA
caatcgccagaacggagaga

SEQ ID NO: 72 - DNA, 20 bp, synthetic construct
  misc_feature 1..20: note = RYR1 Rev
  source 1..20: mol_type = other DNA
gtcgtgttccctgtctgtgt

SEQ ID NO: 73 - DNA, 20 bp, synthetic construct
  misc_feature 1..20: note = SLC17A6 (VGLUT2) Fw
  source 1..20: mol_type = other DNA
gtagactggcaaccacctcc

SEQ ID NO: 74 - DNA, 22 bp, synthetic construct
  misc_feature 1..22: note = SLC17A6 (VGLUT2) Rev
  source 1..22: mol_type = other DNA
ccattccaaagcttccgtagac

SEQ ID NO: 75 - DNA, 22 bp, synthetic construct
  misc_feature 1..22: note = SYP Fw
  source 1..22: mol_type = other DNA
acctcgggactcaacacctcgg

SEQ ID NO: 76 - DNA, 22 bp, synthetic construct
  misc_feature 1..22: note = SYP Rev
  source 1..22: mol_type = other DNA
gaaccacaggttgccgacccag

SEQ ID NO: 77 - DNA, 20 bp, synthetic construct
  misc_feature 1..20: note = SYN1 Fw
  source 1..20: mol_type = other DNA
ccctgggtgtttgcccagat

SEQ ID NO: 78 - DNA, 20 bp, synthetic construct
  misc_feature 1..20: note = SYN1 Rev
  source 1..20: mol_type = other DNA
accacggggtacgttgtact

SEQ ID NO: 79 - DNA, 21 bp, synthetic construct
  misc_feature 1..21: note = TUBB3 Fw
  source 1..21: mol_type = other DNA
caaccagatcggggccaagtt

SEQ ID NO: 80 - DNA, 19 bp, synthetic construct
  misc_feature 1..19: note = TUBB3 Rev
  source 1..19: mol_type = other DNA
ccgagtcgcccacgtagtt

SEQ ID NO: 81 - DNA, 52 bp, synthetic construct
  misc_feature 1..52: note = AAVS1 targeting vector Fw
  source 1..52: mol_type = other DNA
gtgatagagatccctggtgcaggtggactgactcacctgcacctgttttaga

SEQ ID NO: 82 - DNA, 52 bp, synthetic construct
  misc_feature 1..52: note = AAVSI targeting vector Rev
  source 1..52: mol_type = other DNA
actaaaacaggtgcaggtgagtcagtccacctgcaccagggatctctatcac

SEQ ID NO: 83-84 - skipped (2 entries)

SEQ ID NO: 85 - DNA, 268 bp, synthetic construct
  misc_feature 1..268: note = H1 POLIII Promoter H1-TO
  source 1..268: mol_type = other DNA
cgaacgctgacgtcatcaacccgctccaaggaatcgcgggcccagtgtcactaggcgggaacacccagcgcgcgtgcgccctggcaggaagatggctgtgagggacaggggagtggcgccctgcaatatttgcatgtcgctatgtgttctgggaaatcaccataaacgtgaaatgtctttggatttgggaatcttataagttccctatcagtgatagagatccctggtgcaggtggactgactcacctgcacctgttttagagctaga

SEQ ID NO: 86 - DNA, 268 bp, synthetic construct
  misc_feature 1..268: note = H1 POLIII Promoter H1-2TO
  source 1..268: mol_type = other DNA
cgaacgctgacgtcatcaacccgctccaaggaatcgcgggcccagtgtcactaggcgggaacacccagcgcgcgtgcgccctggcaggaagatggctgtgagggacaggggagtggcgccctgcaatatttgcatgtcgctatgtgttctgggaaatcaccataaacgtgaaatccctatcagtgatagagacttataagttccctatcagtgatagagatccctggtgcaggtggactgactcacctgcacctgttttagagctaga